European Patent Specification EP 3 875 486 B1, published April 1, 2026. Title: MONOCLONAL ANTIBODY THAT SPECIFICALLY BINDS TO CD20. Applicant: JSC "BIOCAD". Application PCT/RU2019/050205. The sequence listing filed with the application follows.

SEQUENCE LISTING (8 sequences)

SEQ ID NO: 1 - protein, 451 aa, Artificial sequence BCD132-L-077_HC
EVQLVQPGAEVVKPGASVKVSCKASGYTFTSYNMHWVRQAPGRGLEWMGAIYPGNGDTSYNQKFKGRVTMTRDKSTSTVYMELSSLRSEDTAVYYCARSTYYGGDWYFNVWGQGTLVTVSSASTKGPSVFPLAPSSKSTSGGTAALGCLVKDYFPEPVTVSWNSGALTSGVHTFPAVLQSSGLYSLSSVVTVPSSSLGTQTYICNVNHKPSNTKVDKRVEPKSCDKTHTCPPCPAPELLGGPSVFLFPPKPKDTLMISRTPEVTCVVVDVSHEDPEVKFNWYVDGVEVHNAKTKPREEQYNSTYRVVSVLTVLHQDWLNGKEYKCKVSNKALPAPIEKTISKAKGQPREPQVYTLPPSREEMTKNQVSLTCLVKGFYPSDIAVEWESNGQPENNYKTTPPVLDSDGSFFLYSKLTVDKSRWQQGNVFSCSVMHEALHNHYTQKSLSLSPGK

SEQ ID NO: 2 - protein, 121 aa, Artificial sequence BCD132-L-077_VH
EVQLVQPGAEVVKPGASVKVSCKASGYTFTSYNMHWVRQAPGRGLEWMGAIYPGNGDTSYNQKFKGRVTMTRDKSTSTVYMELSSLRSEDTAVYYCARSTYYGGDWYFNVWGQGTLVTVSS

SEQ ID NO: 3 - protein, 213 aa, Artificial sequence BCD132-L-077_LC
QIVLSQSPAILSASPGERVTLTCRASSSVSYIHWFQQKPGKAPKPLIYATSNLASGVPSRFSGSGSGTDFSLTISRVEPEDFAVYYCQQWTSNPPTFGGGTKVEIKRTVAAPSVFIFPPSDEQLKSGTASVVCLLNNFYPREAKVQWKVDNALQSGNSQESVTEQDSKDSTYSLSSTLTLSKADYEKHKVYACEVTHQGLSSPVTKSFNRGEC

SEQ ID NO: 4 - protein, 106 aa, Artificial sequence BCD132-L-028_HC
QIVLSQSPAILSASPGERVTLTCRASSSVSYIHWFQQKPGKAPKPLIYATSNLASGVPSRFSGSGSGTDFSLTISRVEPEDFAVYYCQQWTSNPPTFGGGTKVEIK

SEQ ID NO: 5 - protein, 451 aa, Artificial sequence BCD132-L-028_HC
QVQLVQSGAEVKKPGASVKVSCKASGYTFTSYNMHWVRQAPGRGLEWMGAIYPGNGDTSYNQKFKGRATLTRDTSTSTVYMELSSLRSEDTAVYYCARSTYYGGDWYFNVWGQGTLVTVSSASTKGPSVFPLAPSSKSTSGGTAALGCLVKDYFPEPVTVSWNSGALTSGVHTFPAVLQSSGLYSLSSVVTVPSSSLGTQTYICNVNHKPSNTKVDKRVEPKSCDKTHTCPPCPAPELLGGPSVFLFPPKPKDTLMISRTPEVTCVVVDVSHEDPEVKFNWYVDGVEVHNAKTKPREEQYNSTYRVVSVLTVLHQDWLNGKEYKCKVSNKALPAPIEKTISKAKGQPREPQVYTLPPSREEMTKNQVSLTCLVKGFYPSDIAVEWESNGQPENNYKTTPPVLDSDGSFFLYSKLTVDKSRWQQGNVFSCSVMHEALHNHYTQKSLSLSPGK

SEQ ID NO: 6 - protein, 121 aa, Artificial sequence BCD132-L-028_VH
QVQLVQSGAEVKKPGASVKVSCKASGYTFTSYNMHWVRQAPGRGLEWMGAIYPGNGDTSYNQKFKGRATLTRDTSTSTVYMELSSLRSEDTAVYYCARSTYYGGDWYFNVWGQGTLVTVSS

SEQ ID NO: 7 - protein, 213 aa, Artificial sequence BCD132-L-028_LC
QIVLSQSPATLSASPGERATMTCRASSSVSYIHWFQQKPGKAPKPLIYATSNLASGVPSRFSGSGSGTDFTLTISRLEPEDFATYYCQQWTSNPPTFGGGTKVEIKRTVAAPSVFIFPPSDEQLKSGTASVVCLLNNFYPREAKVQWKVDNALQSGNSQESVTEQDSKDSTYSLSSTLTLSKADYEKHKVYACEVTHQGLSSPVTKSFNRGEC

SEQ ID NO: 8 - protein, 106 aa, Artificial sequence BCD132-L-028_VL
QIVLSQSPATLSASPGERATMTCRASSSVSYIHWFQQKPGKAPKPLIYATSNLASGVPSRFSGSGSGTDFTLTISRLEPEDFATYYCQQWTSNPPTFGGGTKVEIK